European Patent Specification EP 3 646 877 B1, published December 6, 2023. Title: A composition comprising an exosome from stem cell as an active ingredient and its application for suppressing or improving pruritus. Applicant: ExoCoBio Inc. The sequence listing filed with the application follows.

SEQUENCE LISTING (10 sequences)

SEQ ID NO: 1 - DNA, 19 bp, Artificial Sequence
  IL-4 forward primer
acaggagaagggacgccat

SEQ ID NO: 2 - DNA, 21 bp, Artificial Sequence
  IL-4 reverse primer
gaagccctacagacgagctca

SEQ ID NO: 3 - DNA, 20 bp, Artificial Sequence
  IL-31 forward primer
cacacaggaacaacgaagcc

SEQ ID NO: 4 - DNA, 19 bp, Artificial Sequence
  IL-31 reverse primer
cgatattggggcaccgaag

SEQ ID NO: 5 - DNA, 20 bp, Artificial Sequence
  GAPDH forward primer
catggccttccgtgttccta

SEQ ID NO: 6 - DNA, 22 bp, Artificial Sequence
  GAPDH reverse primer
cctgcttcaccaccttcttgat

SEQ ID NO: 7 - DNA, 21 bp, Artificial Sequence
  TSLP forward primer
gctatctggtgcccaggctat

SEQ ID NO: 8 - DNA, 21 bp, Artificial Sequence
  TSLP reverse primer
cgacgccacaatccttgtaat

SEQ ID NO: 9 - DNA, 20 bp, Artificial Sequence
  beta-actin forward primer
ggccatctcttgctcgaagt

SEQ ID NO: 10 - DNA, 20 bp, Artificial Sequence
  beta-actin reverse primer
gacaccttcaacaccccagc